European Patent Application EP 4 266 056 A1, published October 25, 2023. Title: SIZE-BASED DETECTION AND QUANTIFICATION OF FUNCTIONAL BIO-NANOPARTICLES. Applicant: ATHANOR BIOSCIENCES, INC. The sequence listing filed with the application follows.

SEQUENCE LISTING (4 sequences)

SEQ ID NO: 1 - protein, 15 aa, Artificial Sequence
  Description of Artificial Sequence: Synthetic peptide
GGGGSGGGGSGGGGS

SEQ ID NO: 2 - protein, 14 aa, Artificial Sequence
  Description of Artificial Sequence: Synthetic peptide
GGSGPVGPGGSGAS

SEQ ID NO: 3 - protein, 371 aa, Artificial Sequence
  Description of Artificial Sequence: Synthetic polypeptide
MTSKETFTHYQPQGNSDPAHTATAPGGLSAKAPAMTPLMLDTSSRKLVAWDGTTDGAAVGILAVAADQTSTTLTFYKSGTFRYEDVLWPEAASDETKKRTAFAGTAISIVGGSGPVGPGGSGASQMQLVQSGTEVKKPGESLKISCKGSGYGFITYWIGWVRQMPGKGLEWMGIIYPGDSETRYSPSFQGQVTISADKSINTAYLQWSSLKASDTAIYYCAGGSGISTPMDVWGQGTTVTVSSGGGGSGGGGSGGGGSDIQLTQSPDSLAVSLGERATINCKSSQSVLYSSINKNYLAWYQQKPGQPPKLLIYWASTRESGVPDRFSGSGSGTDFTLTISSLQAEDVAVYYCQQYYSTPYTFGQGTKVEIK

SEQ ID NO: 4 - protein, 711 aa, Artificial Sequence
  Description of Artificial Sequence: Synthetic polypeptide
MTSKETFTHYQPQGNSDPAHTATAPGGLSAKAPAMTPLMLDTSSRKLVAWDGTTDGAAVGILAVAADQTSTTLTFYKSGTFRYEDVLWPEAASDETKKRTAFAGTAISIVGGSGPVGPGGSGASSTIEEQAKTFLDKFNHEAEDLFYQSSLASWNYNTNITEENVQNMNNAGDKWSAFLKEQSTLAQMYPLQEIQNLTVKLQLQALQQNGSSVLSEDKSKRLNTILNTMSTIYSTGKVCNPDNPQECLLLEPGLNEIMANSLDYNERLWAWESWRSEVGKQLRPLYEEYVVLKNEMARANHYEDYGDYWRGDYEVNGVDGYDYSRGQLIEDVEHTFEEIKPLYEHLHAYVRAKLMNAYPSYISPIGCLPAHLLGDMWGRFWTNLYSLTVPFGQKPNIDVTDAMVDQAWDAQRIFKEAEKFFVSVGLPNMTQGFWENSMLTDPGNVQKAVCHPTAWDLGKGDFRILMCTKVTMDDFLTAHHEMGHIQYDMAYAAQPFLLRNGANEGFHEAVGEIMSLSAATPKHLKSIGLLSPDFQEDNETEINFLLKQALTIVGTLPFTYMLEKWRWMVFKGEIPKDQWMKKWWEMKREIVGVVEPVPHDETYCDPASLFHVSNDYSFIRYYTRTLYQFQFQEALCQAAKHEGPLHKCDISNSTEAGQKLFNMLRLGKSEPWTLALENVVGAKNMNVRPLLNYFEPLFTWLKDQNKNSFVG